European Patent Specification EP 3 787 418 B1, published May 29, 2024. Title: Formula with specific beta-lactoglobulin peptides. Applicant: N.V. Nutricia. The sequence listing filed with the application follows.

SEQUENCE LISTING (39 sequences)

SEQ ID NO: 1 - protein, 27 aa, Artificial Sequence
  beta-lactoglobulin peptide fragment
  misc_feature (1)..(1): Xaa can Ile or Leu
XIVTQTMKGLDIQKVAGTWYSLAMAAS

SEQ ID NO: 2 - protein, 32 aa, Artificial Sequence
  beta-lactoglobulin peptide fragment
  misc_feature (1)..(1): Xaa can be Ile or Leu
XIVTQTMKGLDIQKVAGTWYSLAMAASDISLL

SEQ ID NO: 3 - protein, 27 aa, Artificial Sequence
  beta-lactoglobulin peptide fragment
TMKGLDIQKVAGTWYSLAMAASDISLL

SEQ ID NO: 4 - protein, 30 aa, Artificial Sequence
  beta-lactoglobulin peptide fragment
TMKGLDIQKVAGTWYSLAMAASDISLLDAQ

SEQ ID NO: 5 - protein, 32 aa, Artificial Sequence
  beta-lactoglobulin peptide fragment
DIQKVAGTWYSLAMAASDISLLDAQSAPLRVY

SEQ ID NO: 6 - protein, 22 aa, Artificial Sequence
  beta-lactoglobulin peptide fragment
LIVTQTMKGLDIQKVAGTWYSL

SEQ ID NO: 7 - protein, 25 aa, Artificial Sequence
  beta-lactoglobulin peptide fragment
LIVTQTMKGLDIQKVAGTWYSLAMA

SEQ ID NO: 8 - protein, 26 aa, Artificial Sequence
  beta-lactoglobulin peptide fragment
LIVTQTMKGLDIQKVAGTWYSLAMAA

SEQ ID NO: 9 - protein, 27 aa, Artificial Sequence
  beta-lactoglobulin peptide fragment
LIVTQTMKGLDIQKVAGTWYSLAMAAS

SEQ ID NO: 10 - protein, 30 aa, Artificial Sequence
  beta-lactoglobulin peptide fragment
LIVTQTMKGLDIQKVAGTWYSLAMAASDIS

SEQ ID NO: 11 - protein, 32 aa, Artificial Sequence
  beta-lactoglobulin peptide fragment
LIVTQTMKGLDIQKVAGTWYSLAMAASDISLL

SEQ ID NO: 12 - protein, 35 aa, Artificial Sequence
  beta-lactoglobulin peptide fragment
LIVTQTMKGLDIQKVAGTWYSLAMAASDISLLDAQ

SEQ ID NO: 13 - protein, 39 aa, Artificial Sequence
  beta-lactoglobulin peptide fragment
LIVTQTMKGLDIQKVAGTWYSLAMAASDISLLDAQSAPL

SEQ ID NO: 14 - protein, 42 aa, Artificial Sequence
  beta-lactoglobulin peptide fragment
LIVTQTMKGLDIQKVAGTWYSLAMAASDISLLDAQSAPLRVY

SEQ ID NO: 15 - protein, 31 aa, Artificial Sequence
  beta-lactoglobulin peptide fragment
QTMKGLDIQKVAGTWYSLAMAASDISLLDAQ

SEQ ID NO: 16 - protein, 17 aa, Artificial Sequence
  beta-lactoglobulin peptide fragment
AMAASDISLLDAQSAPL

SEQ ID NO: 17 - protein, 17 aa, Artificial Sequence
  beta-lactoglobulin peptide fragment
MAASDISLLDAQSAPLR

SEQ ID NO: 18 - protein, 16 aa, Artificial Sequence
  beta-lactoglobulin peptide fragment
MAASDISLLDAQSAPL

SEQ ID NO: 19 - protein, 19 aa, Artificial Sequence
  beta-lactoglobulin peptide fragment
DIQKVAGTWYSLAMAASDI

SEQ ID NO: 20 - protein, 16 aa, Artificial Sequence
  beta-lactoglobulin peptide fragment
VAGTWYSLAMAASDIS

SEQ ID NO: 21 - protein, 14 aa, Artificial Sequence
  beta-lactoglobulin peptide fragment
GTWYSLAMAASDIS

SEQ ID NO: 22 - protein, 20 aa, Artificial Sequence
  beta-lactoglobulin peptide fragment
DIQKVAGTWYSLAMAASDIS

SEQ ID NO: 23 - protein, 15 aa, Artificial Sequence
  beta-lactoglobulin peptide fragment
VAGTWYSLAMAASDI

SEQ ID NO: 24 - protein, 15 aa, Artificial Sequence
  beta-lactoglobulin peptide fragment
AGTWYSLAMAASDIS

SEQ ID NO: 25 - protein, 13 aa, Artificial Sequence
  beta-lactoglobulin peptide fragment
GTWYSLAMAASDI

SEQ ID NO: 26 - protein, 15 aa, Artificial Sequence
  beta-lactoglobulin peptide fragment
KVAGTWYSLAMAASD

SEQ ID NO: 27 - protein, 15 aa, Artificial Sequence
  beta-lactoglobulin peptide fragment
AASDISLLDAQSAPL

SEQ ID NO: 28 - protein, 15 aa, Artificial Sequence
  beta-lactoglobulin peptide fragment
GTWYSLAMAASDISL

SEQ ID NO: 29 - protein, 15 aa, Artificial Sequence
  beta-lactoglobulin peptide fragment
TWYSLAMAASDISLL

SEQ ID NO: 30 - protein, 15 aa, Artificial Sequence
  beta-lactoglobulin peptide fragment
WYSLAMAASDISLLD

SEQ ID NO: 31 - protein, 15 aa, Artificial Sequence
  beta-lactoglobulin peptide fragment
YSLAMAASDISLLDA

SEQ ID NO: 32 - protein, 15 aa, Artificial Sequence
  beta-lactoglobulin peptide fragment
SDISLLDAQSAPLRV

SEQ ID NO: 33 - protein, 18 aa, Artificial Sequence
  Pepmix peptide 1
QKVAGTWYSLAMAASDIS

SEQ ID NO: 34 - protein, 18 aa, Artificial Sequence
  Pepmix peptide 2
WYSLAMAASDISLLDAQS

SEQ ID NO: 35 - protein, 18 aa, Artificial Sequence
  Pepmix peptide 3
AASDISLLDAQSAPLRVY

SEQ ID NO: 36 - protein, 18 aa, Artificial Sequence
  Pepmix peptide 4
LLDAQSAPLRVYVEELKP

SEQ ID NO: 37 - protein, 27 aa, Artificial Sequence
  beta-lactoglobulin peptide fragment
IIVTQTMKGLDIQKVAGTWYSLAMAAS

SEQ ID NO: 38 - protein, 32 aa, Artificial Sequence
  beta-lactoglobulin peptide fragment
IIVTQTMKGLDIQKVAGTWYSLAMAASDISLL

SEQ ID NO: 39 - protein, 18 aa, Artificial Sequence
  beta-lactoglobulin peptide fragment
AMAASDISLLDAQSAPLR